European Patent Specification EP 3 902 929 B1, published November 13, 2024. Title: FAST AND PORTABLE MICROFLUIDIC DETECTION SYSTEM AS AN ALTERNATIVE TO SALMONELLA'S CLASSICAL CULTURE METHOD. Applicant: TUBITAK. The sequence listing filed with the application follows.

SEQUENCE LISTING (5 sequences)

SEQ ID NO: 1 - DNA, 20 bp, Artificial Sequence
  designed primer/probe
tcgatcagtaccagtcgtct

SEQ ID NO: 2 - DNA, 19 bp, Artificial Sequence
  designed primer/probe
ataccggccttcaaatcgg

SEQ ID NO: 3 - DNA, 40 bp, Artificial Sequence
  designed primer/probe
acaacaaaacccaccgccaggccggggaaattatcgccac

SEQ ID NO: 4 - DNA, 40 bp, Artificial Sequence
  designed primer/probe
accaaaggttcagaacgcgtcgccgggcataccatccaga

SEQ ID NO: 5 - DNA, 19 bp, Artificial Sequence
  designed primer/probe
gtcttatcttgattgaagc